European Patent Application EP 4 137 580 A1, published February 22, 2023. Title: Screening for karyotypes with abberations in the gonosomes by direct quantitative fluorescent PCR. Applicant: Eluthia GmbH. The sequence listing filed with the application follows.

SEQUENCE LISTING (18 sequences)

SEQ ID NO: 1 - DNA, 26 bp, Homo sapiens
gtttctggttttgcctaggtccagtg

SEQ ID NO: 2 - DNA, 21 bp, Homo sapiens
tgacaggtagttttgggtcag

SEQ ID NO: 3 - DNA, 28 bp, Homo sapiens
gtttctgttcttcagactgtagctccac

SEQ ID NO: 4 - DNA, 20 bp, Homo sapiens
gtttctaggcactgtggttc

SEQ ID NO: 5 - DNA, 20 bp, Homo sapiens
aggcgagtagctgtctatga

SEQ ID NO: 6 - DNA, 29 bp, Homo sapiens
gttcttcttttctaccactgaaacagagt

SEQ ID NO: 7 - DNA, 25 bp, Homo sapiens
gatagatgatagagatagatgatag

SEQ ID NO: 8 - DNA, 32 bp, Homo sapiens
gttctttgctcacttttatgtgtgtatgtatc

SEQ ID NO: 9 - DNA, 32 bp, Homo sapiens
cacattttactctaaatcagtccaaatatctc

SEQ ID NO: 10 - DNA, 32 bp, Homo sapiens
gttcttggcaaatcactccatggcacatgtat

SEQ ID NO: 11 - DNA, 20 bp, Homo sapiens
gagcaatgatctcatttgca

SEQ ID NO: 12 - DNA, 31 bp, Homo sapiens
gttcttaagtaaacatgtataggaaaaagct

SEQ ID NO: 13 - DNA, 22 bp, Homo sapiens
agcccattttcataataaatcc

SEQ ID NO: 14 - DNA, 30 bp, Homo sapiens
gttcttaatcagtgctttctgtactattgg

SEQ ID NO: 15 - DNA, 20 bp, Homo sapiens
tggagtctctgggtgaagag

SEQ ID NO: 16 - DNA, 26 bp, Homo sapiens
gttcttcaggagtatgggatcaccag

SEQ ID NO: 17 - DNA, 24 bp, Homo sapiens
agtcatttcctctaacaagtctcc

SEQ ID NO: 18 - DNA, 29 bp, Homo sapiens
gttctttccagagagtcagaatcagtagg